European Patent Specification EP 3 994 183 B1, published June 24, 2026. Title: HYDROGEL COMPOSITIONS AND USES THEREOF. Applicant: Molly Sandra SHOICHET. The sequence listing filed with the application follows.

SEQUENCE LISTING (30 sequences)

SEQ ID NO: 1 - protein, 12 aa, Artificial Sequence
  Synthetic Construct
GRGDSPASSKKG

SEQ ID NO: 2 - protein, 21 aa, Artificial Sequence
  Synthetic Construct
SKAGAGPQGIWGQGAGAKSKS

SEQ ID NO: 3 - DNA, 20 bp, Artificial Sequence
  Synthetic Construct
aaatcattgccaggttttcg

SEQ ID NO: 4 - DNA, 20 bp, Artificial Sequence
  Synthetic Construct
tgccacatggtaaggcataa

SEQ ID NO: 5 - DNA, 17 bp, Artificial Sequence
  Synthetic Construct
gccaacgcgcaggtcta

SEQ ID NO: 6 - DNA, 14 bp, Artificial Sequence
  Synthetic Construct
gccgcagcctcaga

SEQ ID NO: 7 - DNA, 23 bp, Artificial Sequence
  Synthetic Construct
gtcaggcacatcagtaacaaggg

SEQ ID NO: 8 - DNA, 24 bp, Artificial Sequence
  Synthetic Construct
attcagcatctccagcagcaggtc

SEQ ID NO: 9 - DNA, 20 bp, Artificial Sequence
  Synthetic Construct
cctctgacgtccatcgtctc

SEQ ID NO: 10 - DNA, 20 bp, Artificial Sequence
  Synthetic Construct
cggatcttctgctgccgtcg

SEQ ID NO: 11 - DNA, 21 bp, Artificial Sequence
  Synthetic Construct
cgcaagtgtaagaagtgcgaa

SEQ ID NO: 12 - DNA, 25 bp, Artificial Sequence
  Synthetic Construct
cgtagcatttatggagagtgagtct

SEQ ID NO: 13 - DNA, 22 bp, Artificial Sequence
  Synthetic Construct
atctctcggtaccttcgggagc

SEQ ID NO: 14 - DNA, 22 bp, Artificial Sequence
  Synthetic Construct
cctgatgccaccttctaggtcc

SEQ ID NO: 15 - DNA, 20 bp, Artificial Sequence
  Synthetic Construct
ctgcagatggagcatgttgt

SEQ ID NO: 16 - DNA, 20 bp, Artificial Sequence
  Synthetic Construct
tcttcacgaggaggcttgat

SEQ ID NO: 17 - DNA, 20 bp, Artificial Sequence
  Synthetic Construct
atgatgcttggctctggaat

SEQ ID NO: 18 - DNA, 20 bp, Artificial Sequence
  Synthetic Construct
ggtctttgcctgctgagagt

SEQ ID NO: 19 - DNA, 18 bp, Artificial Sequence
  Synthetic Construct
gcggcgagtttccgattt

SEQ ID NO: 20 - DNA, 19 bp, Artificial Sequence
  Synthetic Construct
gctcccgtctccgtttttc

SEQ ID NO: 21 - DNA, 20 bp, Artificial Sequence
  Synthetic Construct
tactcccctgccctcaacaa

SEQ ID NO: 22 - DNA, 20 bp, Artificial Sequence
  Synthetic Construct
catcgctatctgagcagcgc

SEQ ID NO: 23 - DNA, 22 bp, Artificial Sequence
  Synthetic Construct
gaagaacggggctaacaaagat

SEQ ID NO: 24 - DNA, 22 bp, Artificial Sequence
  Synthetic Construct
gtccatatgatccgtgatgtcc

SEQ ID NO: 25 - DNA, 21 bp, Artificial Sequence
  Synthetic Construct
tgcaaggctaccagttacatt

SEQ ID NO: 26 - DNA, 21 bp, Artificial Sequence
  Synthetic Construct
ttagtgttctcaggattggct

SEQ ID NO: 27 - DNA, 19 bp, Artificial Sequence
  Synthetic Construct
tcgtgggctacagcatggt

SEQ ID NO: 28 - DNA, 22 bp, Artificial Sequence
  Synthetic Construct
gccctctgaagtcgaagaagaa

SEQ ID NO: 29 - DNA, 21 bp, Artificial Sequence
  Synthetic Construct
catgtacgttgctatccaggc

SEQ ID NO: 30 - DNA, 21 bp, Artificial Sequence
  Synthetic Construct
ctccttaatgtcacgcacgat